European Patent Application EP 4 483 877 A1, published January 1, 2025. Title: 包含抗CTLA4-抗PD-1双特异性抗体和西奥罗尼的药物组合. Applicant: 康方药业有限公司. The sequence listing filed with the application follows.

SEQUENCE LISTING (44 sequences)

SEQ ID NO: 1 - DNA, 372 bp, synthetic construct
  source 1..372: mol_type = other DNA
caggtcaagctgcaggagtctggacctgagctggtgaagcctggagcttcaatgaagatatcctgcaaggcttctggttactcattcactggctacaccatgaactgggtgaagcagagccatggaaagaaccttgaatggattggacttattaatccttacaataatattactaactacaaccagaagttcatgggcaaggccacatttactgtagacaagtcatccagcacagcctacatggaactcctcagactgacatctgaagactctggagtctatttctgtgcaagactcgactataggtcttattggggccaagggactctggtcactgtctctgcagccaaaacgacacccccatctgtctat

SEQ ID NO: 2 - protein, 124 aa, synthetic construct
QVKLQESGPELVKPGASMKISCKASGYSFTGYTMNWVKQSHGKNLEWIGLINPYNNITNYNQKFMGKATFTVDKSSSTAYMELLRLTSEDSGVYFCARLDYRSYWGQGTLVTVSAAKTTPPSVY

SEQ ID NO: 3 - DNA, 378 bp, synthetic construct
  source 1..378: mol_type = other DNA
caggctgttgtgactcaggaatctgcactcaccacatcacctggtgaaacagtcacactcacttgtcgctcaagtactggggctgttacaactagtaactttgccaactgggtccaagaaaaaccagatcatttattcactagtctaataggtggtaccaacaaccgagctccaggtgttcctgccagattctcaggctccctgattggagacaaggctgccctcaccatcacaggggcacagactgaggatgaggcaatatatttctgtgctctatggtacagcaaccattgggtgttcggtggaggaaccaaactgactgtcctaggccagcccaagtcttcgccatcagtcaccctgtttcaagggcaattctgc

SEQ ID NO: 4 - protein, 126 aa, synthetic construct
QAVVTQESALTTSPGETVTLTCRSSTGAVTTSNFANWVQEKPDHLFTSLIGGTNNRAPGVPARFSGSLIGDKAALTITGAQTEDEAIYFCALWYSNHWVFGGGTKLTVLGQPKSSPSVTLFQGQFC

SEQ ID NO: 5 - DNA, 345 bp, synthetic construct
  source 1..345: mol_type = other DNA
caggtgcagctggtggagtctggggccgagctggtgaagcccggcgcctccatgaagatctcttgcaaggccagcggatacagtttcactggctataccatgaactgggtcaaacaggctccaggacagggactggagtggatcgggctgattaatccttacaacaacatcaccaactacaaccagaagttcatgggaaaagcaacctttacagtggacaagagcatttccacagcctacatggaactgagccggctgacttcagacgatagcggggtctatttttgtgcaaggctggattatcgctcttactgggggcagggaactctggtcactgtctccgct

SEQ ID NO: 6 - protein, 115 aa, synthetic construct
QVQLVESGAELVKPGASMKISCKASGYSFTGYTMNWVKQAPGQGLEWIGLINPYNNITNYNQKFMGKATFTVDKSISTAYMELSRLTSDDSGVYFCARLDYRSYWGQGTLVTVSA

SEQ ID NO: 7 - DNA, 327 bp, synthetic construct
  source 1..327: mol_type = other DNA
caggctgtcgtcactcaggaaccttcactgactgtgagcccaggaggaactgtcaccctgacatgcggaagctccaccggagcagtgaccacatccaacttcgccaattgggtccaggaaaagccaggccaggcatttcgatccctgatcggaggcacaaacaatcgggcttcttgggtgcccgcaagattctcaggaagcctgctggggggaaaagccgctctgaccattagtggcgctcagcctgaggacgaagccgagtacttctgcgctctgtggtatagcaaccactgggtgtttggcgggggaacaaagctgactgtgctg

SEQ ID NO: 8 - protein, 109 aa, synthetic construct
QAVVTQEPSLTVSPGGTVTLTCGSSTGAVTTSNFANWVQEKPGQAFRSLIGGTNNRASWVPARFSGSLLGGKAALTISGAQPEDEAEYFCALWYSNHWVFGGGTKLTVL

SEQ ID NO: 9 - DNA, 345 bp, synthetic construct
  source 1..345: mol_type = other DNA
caggtgcagctggtcgagtctggggccgaagtgaagaaacccggcgcctcagtgaaggtcagctgcaaggccagcgggtacagtttcactggatataccatgaactgggtccgacaggcccctggccaggggctggagtggatcggcctgattaacccttacaacaacatcactaactacgcacagaagttccaggggagagtgacctttacagtggacaccagcatttccacagcctacatggaactgtcccggctgagatctgacgatacaggcgtgtacttctgcgctaggctggattaccgcagctattggggacagggcacactggtgactgtcagcgca

SEQ ID NO: 10 - protein, 115 aa, synthetic construct
QVQLVESGAEVKKPGASVKVSCKASGYSFTGYTMNWVRQAPGQGLEWIGLINPYNNITNYAQKFQGRVTFTVDTSISTAYMELSRLRSDDTGVYFCARLDYRSYWGQGTLVTVSA

SEQ ID NO: 11 - DNA, 327 bp, synthetic construct
  source 1..327: mol_type = other DNA
caggctgtcgtcactcaggaaccttcactgaccgtgtctcctggcgggactgtcaccctgacatgcggcagctccacaggggccgtgaccacaagtaacttcccaaattgggtccagcagaagccaggacaggctccccggagtctgatcggaggcaccaacaacaaggccagctggacacccgcacggttcagcggcagcctgctgggcggcaaggccgctctgacaattagcggagcccagcctgaggacgaagccgagtactattgcgctctgtggtactccaaccactgggtgttcggcggcggcaccaagctgactgtgctg

SEQ ID NO: 12 - protein, 109 aa, synthetic construct
QAVVTQEPSLTVSPGGTVTLTCGSSTGAVTTSNFPNWVQQKPGQAPRSLIGGTNNKASWTPARFSGSLLGGKAALTISGAQPEDEAEYYCALWYSNHWVFGGGTKLTVL

SEQ ID NO: 13 - DNA, 354 bp, synthetic construct
  source 1..354: mol_type = other DNA
gaggtcaaactggtggagagcggcggcgggctggtgaagcccggcgggtcactgaaactgagctgcgccgcttccggcttcgcctttagctcctacgacatgtcatgggtgaggcagacccctgagaagcgcctggaatgggtcgctactatcagcggaggcgggcgatacacctactatcctgactctgtcaaagggagattcacaattagtcgggataacgccagaaatactctgtatctgcagatgtctagtctgcggtccgaggatacagctctgtactattgtgcaaaccggtacggcgaagcatggtttgcctattggggacagggcaccctggtgacagtctctgcc

SEQ ID NO: 14 - protein, 118 aa, synthetic construct
EVKLVESGGGLVKPGGSLKLSCAASGFAFSSYDMSWVRQTPEKRLEWVATISGGGRYTYYPDSVKGRFTISRDNARNTLYLQMSSLRSEDTALYYCANRYGEAWFAYWGQGTLVTVSA

SEQ ID NO: 15 - DNA, 321 bp, synthetic construct
  source 1..321: mol_type = other DNA
gacattaagatgacacagtccccttcctcaatgtacgctagcctgggcgagcgagtgaccttcacatgcaaagcatcccaggacatcaacacatacctgtcttggtttcagcagaagccaggcaaaagccccaagaccctgatctaccgggccaatagactggtggacggggtccccagcagattctccggatctggcagtgggcaggattactccctgaccatcagctccctggagtatgaagacatgggcatctactattgcctgcagtatgatgagttccctctgacctttggagcaggcacaaaactggaactgaag

SEQ ID NO: 16 - protein, 107 aa, synthetic construct
DIKMTQSPSSMYASLGERVTFTCKASQDINTYLSWFQQKPGKSPKTLIYRANRLVDGVPSRFSGSGSGQDYSLTISSLEYEDMGIYYCLQYDEFPLTFGAGTKLELK

SEQ ID NO: 17 - DNA, 354 bp, synthetic construct
  source 1..354: mol_type = other DNA
gaagtgcagctggtcgagtctgggggagggctggtgcagcccggcgggtcactgcgactgagctgcgcagcttccggattcgcctttagctcctacgacatgtcctgggtgcgacaggcaccaggaaagggactggattgggtcgctactatctcaggaggcgggagatacacctactatcctgacagcgtcaagggccggttcacaatctctagagataacagtaagaacaatctgtatctgcagatgaacagcctgagggctgaggacaccgcactgtactattgtgccaaccgctacggggaagcatggtttgcctattgggggcagggaaccctggtgacagtctctagt

SEQ ID NO: 18 - protein, 118 aa, synthetic construct
EVQLVESGGGLVQPGGSLRLSCAASGFAFSSYDMSWVRQAPGKGLDWVATISGGGRYTYYPDSVKGRFTISRDNSKNNLYLQMNSLRAEDTALYYCANRYGEAWFAYWGQGTLVTVSS

SEQ ID NO: 19 - DNA, 321 bp, synthetic construct
  source 1..321: mol_type = other DNA
gacattcagatgactcagagcccctcctccatgtccgcctctgtgggcgacagggtcaccttcacatgccgcgctagtcaggatatcaacacctacctgagctggtttcagcagaagccagggaaaagccccaagacactgatctaccgggctaatagactggtgtctggagtcccaagtcggttcagtggctcagggagcggacaggactacactctgaccatcagctccctgcagcctgaggacatggcaacctactattgcctgcagtatgatgagttcccactgacctttggcgccgggacaaaactggagctgaag

SEQ ID NO: 20 - protein, 107 aa, synthetic construct
DIQMTQSPSSMSASVGDRVTFTCRASQDINTYLSWFQQKPGKSPKTLIYRANRLVSGVPSRFSGSGSGQDYTLTISSLQPEDMATYYCLQYDEFPLTFGAGTKLELK

SEQ ID NO: 21 - DNA, 1344 bp, synthetic construct
  source 1..1344: mol_type = other DNA
gaagtgcagctggtcgagtctgggggagggctggtgcagcccggcgggtcactgcgactgagctgcgcagcttccggattcgcctttagctcctacgacatgtcctgggtgcgacaggcaccaggaaagggactggattgggtcgctactatctcaggaggcgggagatacacctactatcctgacagcgtcaagggccggttcacaatctctagagataacagtaagaacaatctgtatctgcagatgaacagcctgagggctgaggacaccgcactgtactattgtgccaaccgctacggggaagcatggtttgcctattgggggcagggaaccctggtgacagtctctagtgccagcaccaaaggacctagcgtgtttcctctcgccccctcctccaaaagcaccagcggaggaaccgctgctctcggatgtctggtgaaggactacttccctgaacccgtcaccgtgagctggaatagcggcgctctgacaagcggagtccatacattccctgctgtgctgcaaagcagcggactctattccctgtccagcgtcgtcacagtgcccagcagcagcctgggcacccagacctacatctgtaacgtcaaccacaagccctccaacaccaaggtggacaagaaagtggagcccaaatcctgcgacaagacacacacctgtcccccctgtcctgctcccgaactcctcggaggccctagcgtcttcctctttcctcccaaacccaaggacaccctcatgatcagcagaacccctgaagtcacctgtgtcgtcgtggatgtcagccatgaggaccccgaggtgaaattcaactggtatgtcgatggcgtcgaggtgcacaacgccaaaaccaagcccagggaggaacagtacaactccacctacagggtggtgtccgtgctgacagtcctccaccaggactggctgaacggcaaggagtacaagtgcaaggtgtccaacaaggctctccctgcccccattgagaagaccatcagcaaggccaaaggccaacccagggagccccaggtctatacactgcctccctccagggacgaactcaccaagaaccaggtgtccctgacctgcctggtcaagggcttttatcccagcgacatcgccgtcgagtgggagtccaacggacagcccgagaataactacaagaccacccctcctgtcctcgactccgacggctccttcttcctgtacagcaagctgaccgtggacaaaagcaggtggcagcagggaaacgtgttctcctgcagcgtgatgcacgaagccctccacaaccactacacccagaaaagcctgtccctgagccccggcaaa

SEQ ID NO: 22 - protein, 448 aa, synthetic construct
EVQLVESGGGLVQPGGSLRLSCAASGFAFSSYDMSWVRQAPGKGLDWVATISGGGRYTYYPDSVKGRFTISRDNSKNNLYLQMNSLRAEDTALYYCANRYGEAWFAYWGQGTLVTVSSASTKGPSVFPLAPSSKSTSGGTAALGCLVKDYFPEPVTVSWNSGALTSGVHTFPAVLQSSGLYSLSSVVTVPSSSLGTQTYICNVNHKPSNTKVDKKVEPKSCDKTHTCPPCPAPELLGGPSVFLFPPKPKDTLMISRTPEVTCVVVDVSHEDPEVKFNWYVDGVEVHNAKTKPREEQYNSTYRVVSVLTVLHQDWLNGKEYKCKVSNKALPAPIEKTISKAKGQPREPQVYTLPPSRDELTKNQVSLTCLVKGFYPSDIAVEWESNGQPENNYKTTPPVLDSDGSFFLYSKLTVDKSRWQQGNVFSCSVMHEALHNHYTQKSLSLSPGK

SEQ ID NO: 23 - DNA, 642 bp, synthetic construct
  source 1..642: mol_type = other DNA
gacattcagatgactcagagcccctcctccatgtccgcctctgtgggcgacagggtcaccttcacatgccgcgctagtcaggatatcaacacctacctgagctggtttcagcagaagccagggaaaagccccaagacactgatctaccgggctaatagactggtgtctggagtcccaagtcggttcagtggctcagggagcggacaggactacactctgaccatcagctccctgcagcctgaggacatggcaacctactattgcctgcagtatgatgagttcccactgacctttggcgccgggacaaaactggagctgaagcgaactgtggccgctccctccgtcttcatttttcccccttctgacgaacagctgaaatcaggcacagccagcgtggtctgtctgctgaacaatttctaccctagagaggcaaaagtgcagtggaaggtcgataacgccctgcagtccggcaacagccaggagagtgtgactgaacaggactcaaaagatagcacctattccctgtctagtacactgactctgtccaaggctgattacgagaagcacaaagtgtatgcatgcgaagtgacacatcagggactgtcaagccccgtgactaagtcttttaaccggggcgaatgt

SEQ ID NO: 24 - protein, 214 aa, synthetic construct
DIQMTQSPSSMSASVGDRVTFTCRASQDINTYLSWFQQKPGKSPKTLIYRANRLVSGVPSRFSGSGSGQDYTLTISSLQPEDMATYYCLQYDEFPLTFGAGTKLELKRTVAAPSVFIFPPSDEQLKSGTASVVCLLNNFYPREAKVQWKVDNALQSGNSQESVTEQDSKDSTYSLSSTLTLSKADYEKHKVYACEVTHQGLSSPVTKSFNRGEC

SEQ ID NO: 25 - protein, 15 aa, synthetic construct
GGGGSGGGGSGGGGS

SEQ ID NO: 26 - protein, 20 aa, synthetic construct
GGGGSGGGGSGGGGSGGGGS

SEQ ID NO: 27 - protein, 8 aa, synthetic construct
GFAFSSYD

SEQ ID NO: 28 - protein, 8 aa, synthetic construct
ISGGGRYT

SEQ ID NO: 29 - protein, 11 aa, synthetic construct
ANRYGEAWFAY

SEQ ID NO: 30 - protein, 6 aa, synthetic construct
QDINTY

SEQ ID NO: 31 - skipped

SEQ ID NO: 32 - protein, 9 aa, synthetic construct
LQYDEFPLT

SEQ ID NO: 33 - protein, 8 aa, synthetic construct
GYSFTGYT

SEQ ID NO: 34 - protein, 8 aa, synthetic construct
INPYNNIT

SEQ ID NO: 35 - protein, 8 aa, synthetic construct
ARLDYRSY

SEQ ID NO: 36 - protein, 9 aa, synthetic construct
TGAVTTSNF

SEQ ID NO: 37 - skipped

SEQ ID NO: 38 - protein, 9 aa, synthetic construct
ALWYSNHWV

SEQ ID NO: 39 - DNA, 1344 bp, synthetic construct
  source 1..1344: mol_type = other DNA
gaagtgcagctggtcgagtctgggggagggctggtgcagcccggcgggtcactgcgactgagctgcgcagcttccggattcgcctttagctcctacgacatgtcctgggtgcgacaggcaccaggaaagggactggattgggtcgctactatctcaggaggcgggagatacacctactatcctgacagcgtcaagggccggttcacaatctctagagataacagtaagaacaatctgtatctgcagatgaacagcctgagggctgaggacaccgcactgtactattgtgccaaccgctacggggaagcatggtttgcctattgggggcagggaaccctggtgacagtctctagtgccagcaccaaagggcccagcgtgtttcctctcgccccctcctccaaaagcaccagcggaggaaccgctgctctcggatgtctggtgaaggactacttccctgaacccgtcaccgtgagctggaatagcggcgctctgacaagcggagtccatacattccctgctgtgctgcaaagcagcggactctattccctgtccagcgtcgtcacagtgcccagcagcagcctgggcacccagacctacatctgtaacgtcaaccacaagccctccaacaccaaggtggacaagaaagtggagcccaaatcctgcgacaagacacacacctgtcccccctgtcctgctcccgaagctgctggagcccctagcgtcttcctctttcctcccaaacccaaggacaccctcatgatcagcagaacccctgaagtcacctgtgtcgtcgtggatgtcagccatgaggaccccgaggtgaaattcaactggtatgtcgatggcgtcgaggtgcacaacgccaaaaccaagcccagggaggaacagtacaactccacctacagggtggtgtccgtgctgacagtcctccaccaggactggctgaacggcaaggagtacaagtgcaaggtgtccaacaaggctctccctgcccccattgagaagaccatcagcaaggccaaaggccaacccagggagccccaggtctatacactgcctccctccagggacgaactcaccaagaaccaggtgtccctgacctgcctggtcaagggcttttatcccagcgacatcgccgtcgagtgggagtccaacggacagcccgagaataactacaagaccacccctcctgtcctcgactccgacggctccttcttcctgtacagcaagctgaccgtggacaaaagcaggtggcagcagggaaacgtgttctcctgcagcgtgatgcacgaagccctccacaaccactacacccagaaaagcctgtccctgagccccggcaaa

SEQ ID NO: 40 - protein, 448 aa, synthetic construct
EVQLVESGGGLVQPGGSLRLSCAASGFAFSSYDMSWVRQAPGKGLDWVATISGGGRYTYYPDSVKGRFTISRDNSKNNLYLQMNSLRAEDTALYYCANRYGEAWFAYWGQGTLVTVSSASTKGPSVFPLAPSSKSTSGGTAALGCLVKDYFPEPVTVSWNSGALTSGVHTFPAVLQSSGLYSLSSVVTVPSSSLGTQTYICNVNHKPSNTKVDKKVEPKSCDKTHTCPPCPAPEAAGAPSVFLFPPKPKDTLMISRTPEVTCVVVDVSHEDPEVKFNWYVDGVEVHNAKTKPREEQYNSTYRVVSVLTVLHQDWLNGKEYKCKVSNKALPAPIEKTISKAKGQPREPQVYTLPPSRDELTKNQVSLTCLVKGFYPSDIAVEWESNGQPENNYKTTPPVLDSDGSFFLYSKLTVDKSRWQQGNVFSCSVMHEALHNHYTQKSLSLSPGK

SEQ ID NO: 41 - protein, 115 aa, synthetic construct
QVQLVESGAELVKPGASMKISCKASGYSFTGYTMNWVKQAPGQCLEWIGLINPYNNITNYNQKFMGKATFTVDKSISTAYMELSRLTSDDSGVYFCARLDYRSYWGQGTLVTVSA

SEQ ID NO: 42 - protein, 110 aa, synthetic construct
QAVVTQEPSLTVSPGGTVTLTCGSSTGAVTTSNFANWVQEKPGQAFRSLIGGTNNRASWVPARFSGSLLGGKAALTISGAQPEDEAEYFCALWYSNHWVFGCGTKLTVLR

SEQ ID NO: 43 - protein, 115 aa, synthetic construct
QVQLVESGAEVKKPGASVKVSCKASGYSFTGYTMNWVRQAPGQCLEWIGLINPYNNITNYAQKFQGRVTFTVDTSISTAYMELSRLRSDDTGVYFCARLDYRSYWGQGTLVTVSA

SEQ ID NO: 44 - protein, 110 aa, synthetic construct
QAVVTQEPSLTVSPGGTVTLTCGSSTGAVTTSNFPNWVQQKPGQAPRSLIGGTNNKASWTPARFSGSLLGGKAALTISGAQPEDEAEYYCALWYSNHWVFGCGTKLTVLR